European Patent Specification EP 3 390 442 B1, published November 8, 2023. Title: ANTI-C5 ANTIBODIES AND METHODS OF USE. Applicant: CHUGAI SEIYAKU KABUSHIKI KAISHA. The sequence listing filed with the application follows.

SEQUENCE LISTING (150 sequences)

SEQ ID NO: 1 - protein, 121 aa, Artificial sequence
  An artificially synthesized sequence
QSLEESGGDLVKPGASLAVTCTASGFSSSSSYYMCWVRQAPGKGLEWIGCIYTGSGATYYASWAKGRFTISKTSSTTVTLQMTSLTVADTATYFCASDGGYVTPTHAMYLWGPGTLVTVSS

SEQ ID NO: 2 - protein, 117 aa, Artificial sequence
  An artificially synthesized sequence
QSLEESGGGLVKPGASLTLTCKASGIDFSNFYYICWVRQAPGKGLDLIACIYTVSGYTYYASWAKGRLTISKTSSTTVTLQMTSLTAADTATYFCARDLHAGITNLWGPGTLVTVSS

SEQ ID NO: 3 - protein, 122 aa, Artificial sequence
  An artificially synthesized sequence
QSLEESGGDLVKPGASLSLTCTAAGLDFSSSYYMCWVRQAPGKGLEWIACIYAGSSGIIYYANWAKGRFTISRPSSTTVTLQMTSLTAADTATYFCATYPTYGDGGHAFNLWGPGTLVTVSS

SEQ ID NO: 4 - protein, 117 aa, Artificial sequence
  An artificially synthesized sequence
QSVEESGGRLVTPGTPLTLTCTASGFSLSSYYMNWVRQAPGKGLEWIGMIYGSGATYYASWAKGRFTISKTSSTTVDLKMTSLTTEDTATYFCARQIYSGDNNDNFWGPGTLVTVSS

SEQ ID NO: 5 - protein, 117 aa, Artificial sequence; identical to SEQ ID NO: 4
  An artificially synthesized sequence

SEQ ID NO: 6 - protein, 117 aa, Artificial sequence
  An artificially synthesized sequence
QSVEESGGRLVTPGTPLTLTCTVSGLSLSDNTMTWVRQAPGKGLEWIGIISFGGDAYYASWAKGRFPISKTSTTVDLRITSPTTEDTATYFCARVGAGNIFWYFDLWGPGTLVTVSS

SEQ ID NO: 7 - protein, 116 aa, Artificial sequence
  An artificially synthesized sequence
QSVEESGGRLVTPGTPLTLTCTVSGFSLSTYAMGWVRQAPGKGLEWIGTIDTGDNSFYANWAKGRFTISKTSTTVDLKITSPTAEDTATYFCARNDGSVYNLFNLWGPGTLVTVSS

SEQ ID NO: 8 - protein, 110 aa, Artificial sequence
  An artificially synthesized sequence
QSVEESGGRLVTPGTPLTLTCTASGFSLSGNAINWVRQAPGKGLEWIGCIYTGSDTTYYATWAKGRFTISKTSTTVDLKIASPTTEDTATYFCARGSGLWGPGTLVTVSS

SEQ ID NO: 9 - protein, 116 aa, Artificial sequence
  An artificially synthesized sequence
QSVEESGGRLVTPGTPLTLTCTVSGFSLSTYAMGWVRQAPGKGLEWIGTIDTGDNSFYANWAKGRFTISRTSTTVDLKITSPTAEDTATYFCARNDGSVYNLFNLWGPGTLVTVSS

SEQ ID NO: 10 - protein, 123 aa, Artificial sequence
  An artificially synthesized sequence
QVQLVESGGGLVQPGGSLRLSCAASGFTSHSSYYVAWVRQAPGKGLEWVGAIYTGSGATYKASWAKGRFTISKDTSKNQVVLTMTNMDPVDTATYYCASDGGYDYPTHAMHYWGQGTLVTVSS

SEQ ID NO: 11 - protein, 110 aa, Artificial sequence
  An artificially synthesized sequence
DVVMTQTPASVSAAVGGTVTIKCQASQNIGSDLAWYQQKPGQPPRLLIYGASKLASGVSSRFSGSGSGKEFTLTISDLECADAVTYYCQCTFVGSSYGNAFGGGTEVVVK

SEQ ID NO: 12 - protein, 110 aa, Artificial sequence
  An artificially synthesized sequence
AIEMTQTPFSVSAAVGGTVTIKCQASQNIYSNLAWYQQKPGQRPKLLIYGASNLESGVPSRFKGSGSGTEYTLTISDLECADAATYYCLQGYSYSNVDDAFGGGTEVVVK

SEQ ID NO: 13 - protein, 112 aa, Artificial sequence
  An artificially synthesized sequence
AQVLTQTPSSVSAAVGGTVTINCQSSQSVYSSDYLSWYQQKPGQPPKLLIYEASKLASGVPPRFSGSGSGTQFTLTISGVQCDDAATYYCQGTYYSSGWYFAFGGGTEVVVK

SEQ ID NO: 14 - protein, 110 aa, Artificial sequence
  An artificially synthesized sequence
AYDMTQTPASVEVAVGGTVTINCQASESISNWLAWYQQKPGQRPKLLIYRASTLASGVSSRFKGSGSGTQFTLTISGVECDDAATYYCQQDYSSSNVDNTFGGGTKVVVE

SEQ ID NO: 15 - protein, 110 aa, Artificial sequence
  An artificially synthesized sequence
AYDMTQTPASVEVAVGGTVTINCQASESISNWLAWYQQKPGQRPKLLIYRASTLASGVSSRFKGSGSGTQFTLTISGVECDDAATYYCQQDYSSSNVDNTFGGGTTVVVE

SEQ ID NO: 16 - protein, 110 aa, Artificial sequence
  An artificially synthesized sequence
AYDMTQTPASVEVSVGGTVTIKCQASESIYSALAWYQQKPGQPPKLLIYSASTLASGVPSRFKGSGSGTEYTLTISDLECADAATYYCQQYYSSTNVHNSFGGGTTVVVE

SEQ ID NO: 17 - protein, 110 aa, Artificial sequence
  An artificially synthesized sequence
DVVMTQTPASVSAAVGGTVTIKCQASENIYSALSWYQQKPGLRPRLLIYYASTLASGVPSRFKGSRSGTEFTLTISDLECADAATYYCQQYYDINSVDNTFGGGTKVVVE

SEQ ID NO: 18 - protein, 111 aa, Artificial sequence
  An artificially synthesized sequence
DVVMTQTPASVSAPVGGTVTIKCQASQNIYSLLAWYQQKPGQPPKLLIYHTSDLASGVPSRFRGSGSGTEFTLTISDLECADAATYYCQCTAYGSSDVGGTFGGGTTVVVE

SEQ ID NO: 19 - protein, 110 aa, Artificial sequence
  An artificially synthesized sequence
DVVMTQTPASVSAAVGGTVTIKCQASENIYSALSWYQQKPGLRPRLLIYYASTLASGVPSRFKGSRSGTEFTLTISDLECADAASYYCQQYYDINSVDNTFGGGTKVVVE

SEQ ID NO: 20 - protein, 110 aa, Artificial sequence
  An artificially synthesized sequence
DVVMTQSPSSLSASVGDRVTITCQASQNIGSSLAWYQQKPGQAPRLLIYGASKTHSGVPSRFSGSGSGTDFTLTISSLQPEDVATYYCQSTKVGSSYGNHFGGGTKVEIK

SEQ ID NO: 21 - protein, 117 aa, Artificial sequence
  An artificially synthesized sequence
QSLEESGGDLVEPGASLTLTCTASGFSWNSGYDMCWVRQAPGKGLEWIACIYTGSSANTAYANWAKGRFTISKTSSTTVTLQMTGLTAADTATYFCARHDDYFFDLWGPGTLVTVSS

SEQ ID NO: 22 - protein, 115 aa, Artificial sequence
  An artificially synthesized sequence
QSVEESGGRLVTPGTPLTLTCTVSGIDLSSYTMGWVRQAPGKGLECIGYIHSFGSTYYASWAKGRFTISKTSTTVDLEITSPTTEDTATYFCARDVGGSSGWDLWGQGTLVTVSS

SEQ ID NO: 23 - protein, 116 aa, Artificial sequence
  An artificially synthesized sequence
QSLEESGGGLVKPGASLTLTCTASGFSFSSGYYMCWVRQAPGKGLEWIGCIGTISDSTYYASWAKGRFPISKASSTTVTLQMTSLTAADTATYFCARDPYSYGDLWGPGTLVTVSS

SEQ ID NO: 24 - protein, 125 aa, Artificial sequence
  An artificially synthesized sequence
QEQLEESGGDLVKPEGSLTLTCTASGFSFSSGNWICWVRQAPGKGLEWIACIYGGSVGGTDYASWAKGRFTVSKTSSTTVTLQMTSLTAADTATYFCARMEDGYGYGYDTYFKLWGPGTLVTVSS

SEQ ID NO: 25 - protein, 114 aa, Artificial sequence
  An artificially synthesized sequence
DVVMTQTPASVSESVGGTVTINCQASQSIGNNLAWYQQKPGQPPKLLIYDASNLASGVPSRFKGSRSGTEPTLTNTLTISGVQCADVATYYCQSGWYGNSYVAAFGGGTEVVVK

SEQ ID NO: 26 - protein, 112 aa, Artificial sequence
  An artificially synthesized sequence
DVVMTQTPSSVSAAVGGTVTIKCQASENIYSNLAWYQQKPGQPPKRLIYDASDLASGVPSRFSGSGYGTQFTLTISGVQCEDAATYYCQANYDSTSSSFGNVFGGGTEVVVK

SEQ ID NO: 27 - protein, 110 aa, Artificial sequence
  An artificially synthesized sequence
DLVMTQTPASVSEPVGGTVTIKCQASQSIGTYLAWYQQKPGQPPKLLIYRASTLASGVPSRFKGSGSGTQFTLTISDLECADAATYYCLGGYYGFSYGNAFGGGTEVVVK

SEQ ID NO: 28 - protein, 110 aa, Artificial sequence
  An artificially synthesized sequence
DIVMTQTPASVEAAVGGTVTIKCQASQSITSWLAWYQQKLGQPPKLLIYKASTLASGVSSRFKGSGSGTEFTLTISDLECADAATYYCQGYYDSSTSSYVFGGGTEVVVK

SEQ ID NO: 29 - protein, 448 aa, Artificial sequence
  An artificially synthesized sequence
QVQLVQSGAEVKKPGASVKVSCKASGYIFSNYWIQWVRQAPGQGLEWMGEILPGSGSTEYTENFKDRVTMTRDTSTSTVYMELSSLRSEDTAVYYCARYFFGSSPNWYFDVWGQGTLVTVSSASTKGPSVFPLAPCSRSTSESTAALGCLVKDYFPEPVTVSWNSGALTSGVHTFPAVLQSSGLYSLSSVVTVPSSNFGTQTYTCNVDHKPSNTKVDKTVERKCCVECPPCPAPPVAGPSVFLFPPKPKDTLMISRTPEVTCVVVDVSQEDPEVQFNWYVDGVEVHNAKTKPREEQFNSTYRVVSVLTVLHQDWLNGKEYKCKVSNKGLPSSIEKTISKAKGQPREPQVYTLPPSQEEMTKNQVSLTCLVKGFYPSDIAVEWESNGQPENNYKTTPPVLDSDGSFFLYSRLTVDKSRWQEGNVFSCSVMHEALHNHYTQKSLSLSLGK

SEQ ID NO: 30 - protein, 214 aa, Artificial sequence [sequence omitted]

SEQ ID NO: 31 - protein, 122 aa, Artificial sequence [sequence omitted]

SEQ ID NO: 32 - protein, 107 aa, Artificial sequence [sequence omitted]

SEQ ID NO: 33 - protein, 325 aa, Artificial sequence
  An artificially synthesized sequence
ASTKGPSVFPLAPCSRSTSESTAALGCLVKDYFPEPVTVSWNSGALTSGVHTFPAVLQSSGLYSLSSVVTVPSSSLGTKTYTCNVDHKPSNTKVDKRVESKYGPPCPPCPAPEFRGGPKVFLFPPKPKDTLMISRTPEVTCVVVDVSQEDPEVQFNWYVDGVEVHNAKTKPREEQFNSTYRVVSVLTVLHQDWLNGKEYKCKVSNKGLPSSIEKTISKAKGQPREPQVYTLPPSQEEMTKNQVSLTCLVKGFYPSDIAVEWESNGQPENNYKTTPPVLDSDGSFFLYSRLTVDKSRWQEGNVFSCSVMHEALHNHYTQKSLSLSL

SEQ ID NO: 34 - protein, 325 aa, Artificial sequence
  An artificially synthesized sequence
ASTKGPSVFPLAPCSRSTSESTAALGCLVKDYFPEPVTVSWNSGALTSGVHTFPAVLQSSGLYSLSSVVTVPSSSLGTKTYTCNVDHKPSNTKVDKRVESKYGPPCPPCPAPEFRGGPKVFLFPPKPKDTLYISRTPEVTCVVVDVSQEDPEVQFNWYVDGVEVHNAKTKPREEQFNSTYRVVSVLTVLHQDWLNGKEYKCKVSNKGLPSSIEKTISKAKGQPREPQVYTLPPSQEEMTKNQVSLTCLVKGFYPSDIAVEWESNGQPENNYKTTPPVLDSDGSFFLYSRLTVDKSRWQEGNVFSCSVMHEALHYHVTQKSLSLSL

SEQ ID NO: 35 - protein, 325 aa, Artificial sequence
  An artificially synthesized sequence
ASTKGPSVFPLAPCSRSTSESTAALGCLVKDYFPEPVTVSWNSGALTSGVHTFPAVLQSSGLYSLSSVVTVPSSSLGTKTYTCNVDHKPSNTKVDKRVESKYGPPCPPCPAPEFRGGPKVFLFPPKPKDTLMISRTPEVTCVVVDVSQEDPEVQFNWYVDGVEVHNAKTKPREEQFNSTYRVVSVLTVLHQDWLNGKEYKCKVSNKGLPSSIEKTISKAKGQPREPQVYTLPPSQEEMTKNQVSLTCLVKGFYPSDIAVEWESNGQPENNYKTTPPVLDSDGSFFLYSKLTVDKSRWQEGNVFSCSVMHEALHNHYTQKSLSLSP

SEQ ID NO: 36 - protein, 107 aa, Artificial sequence
  An artificially synthesized sequence
RTVAAPSVFIFPPSDEQLKSGTASVVCLLNNFYPREAKVQWKVDNALQSGNSQESVTEQDSKDCTYSLSSTLTLSKADYEKHKVYACEVTHQGLSSPVTKSFNRGEC

SEQ ID NO: 37 - protein, 107 aa, Artificial sequence [sequence omitted]

SEQ ID NO: 38 - protein, 107 aa, Artificial sequence [sequence omitted]

SEQ ID NO: 39 - protein, 1676 aa, Homo sapiens
MGLLGILCFLIFLGKTWGQEQTYVISAPKIFRVGASENIVIQVYGYTEAFDATISIKSYPDKKFSYSSGHVHLSSENKFQNSAILTIQPKQLPGGQNPVSYVYLEVVSKHFSKSKRMPITYDNGFLFIHTDKPVYTPDQSVKVRVYSLNDDLKPAKRETVLTFIDPEGSEVDMVEEIDHIGIISFPDFKIPSNPRYGMWTIKAKYKEDFSTTGTAYFEVKEYVLPHFSVSIEPEYNFIGYKNFKNFEITIKARYFYNKVVTEADVYITFGIREDLKDDQKEMMQTAMQNTMLINGIAQVTFDSETAVKELSYYSLEDLNNKYLYIAVTVIESTGGFSEEAEIPGIKYVLSPYKLNLVATPLFLKPGIPYPIKVQVKDSLDQLVGGVPVTLNAQTIDVNQETSDLDPSKSVTRVDDGVASFVLNLPSGVTVLEFNVKTDAPDLPEENQAREGYRAIAYSSLSQSYLYIDWTDNHKALLVGEHLNIIVTPKSPYIDKITHYNYLILSKGKIIHFGTREKFSDASYQSINIPVTQNMVPSSRLLVYYIVTGEQTAELVSDSVWLNIEEKCGNQLQVHLSPDADAYSPGQTVSLNMATGMDSWVALAAVDSAVYGVQRGAKKPLERVFQFLEKSDLGCGAGGGLNNANVFHLAGLTFLTNANADDSQENDEPCKEILRPRRTLQKKIEEIAAKYKHSVVKKCCYDGACVNNDETCEQRAARISLGPRCIKAFTECCVVASQLRANISHKDMQLGRLHMKTLLPVSKPEIRSYFPESWLWEVHLVPRRKQLQFALPDSLTTWEIQGVGISNTGICVADTVKAKVFKDVFLEMNIPYSVVRGEQIQLKGTVYNYRTSGMQFCVKMSAVEGICTSESPVIDHQGTKSSKCVRQKVEGSSSHLVTFTVLPLEIGLHNINFSLETWFGKEILVKTLRVVPEGVKRESYSGVTLDPRGIYGTISRRKEFPYRIPLDLVPKTEIKRILSVKGLLVGEILSAVLSQEGINILTHLPKGSAEAELMSVVPVFYVFHYLETGNHWNIFHSDPLIEKQKLKKKLKEGMLSIMSYRNADYSYSVWKGGSASTWLTAFALRVLGQVNKYVEQNQNSICNSLLWLVENYQLDNGSFKENSQYQPIKLQGTLPVEARENSLYLTAFTVIGIRKAFDICPLVKIDTALIKADNFLLENTLPAQSTFTLAISAYALSLGDKTHPQFRSIVSALKREALVKGNPPIYRFWKDNLQHKDSSVPNTGTARMVETTAYALLTSLNLKDINYVNPVIKWLSEEQRYGGGFYSTQDTINAIEGLTEYSLLVKQLRLSMDIDVSYKHKGALHNYKMTDKNFLGRPVEVLLNDDLIVSTGFGSGLATVHVTTVVHKTSTSEEVCSFYLKIDTQDIEASHYRGYGNSDYKRIVACASYKPSREESSSGSSHAVMDISLPTGISANEEDLKALVEGVDQLFTDYQIKDGHVILQLNSIPSSDFLCVRFRIFELFEVGFLSPATFTVYEYHRPDKQCTMFYSTSNIKIQKVCEGAACKCVEADCGQMQEELDLTISAETRKQTACKPEIAYAYKVSITSITVENVFVKYKATLLDIYKTGEAVAEKDSEITFIKKVTCTNAELVKGRQYLIMGKEALQIKYNFSFRYIYPLDSLTWIEYWPRDTTCSSCQAFLANLDEFAEDIFLNGC

SEQ ID NO: 40 - protein, 673 aa, Homo sapiens
MGLLGILCFLIFLGKTWGQEQTYVISAPKIFRVGASENIVIQVYGYTEAFDATISIKSYPDKKFSYSSGHVHLSSENKFQNSAILTIQPKQLPGGQNPVSYVYLEVVSKHFSKSKRMPITYDNGFLFIHTDKPVYTPDQSVKVRVYSLNDDLKPAKRETVLTFIDPEGSEVDMVEEIDHIGIISFPDFKIPSNPRYGMWTIKAKYKEDFSTTGTAYFEVKEYVLPHFSVSIEPEYNFIGYKNFKNFEITIKARYFYNKVVTEADVYITFGIREDLKDDQKEMMQTAMQNTMLINGIAQVTFDSETAVKELSYYSLEDLNNKYLYIAVTVIESTGGFSEEAEIPGIKYVLSPYKLNLVATPLFLKPGIPYPIKVQVKDSLDQLVGGVPVTLNAQTIDVNQETSDLDPSKSVTRVDDGVASFVLNLPSGVTVLEFNVKTDAPDLPEENQAREGYRAIAYSSLSQSYLYIDWTDNHKALLVGEHLNIIVTPKSPYIDKITHYNYLILSKGKIIHFGTREKFSDASYQSINIPVTQNMVPSSRLLVYYIVTGEQTAELVSDSVWLNIEEKCGNQLQVHLSPDADAYSPGQTVSLNMATGMDSWVALAAVDSAVYGVQRGAKKPLERVFQFLEKSDLGCGAGGGLNNANVFHLAGLTFLTNANADDSQENDEPCKEIL

SEQ ID NO: 41 - protein, 105 aa, Homo sapiens
EQTYVISAPKIFRVGASENIVIQVYGYTEAFDATISIKSYPDKKFSYSSGHVHLSSENKFQNSAILTIQPKQLPGGQNPVSYVYLEVVSKHFSKSKRMPITYDNG

SEQ ID NO: 42 - protein, 101 aa, Homo sapiens
FLFIHTDKPVYTPDQSVKVRVYSLNDDLKPAKRETVLTFIDPEGSEVDMVEEIDHIGIISFPDFKIPSNPRYGMWTIKAKYKEDFSTTGTAYFEVKEYVLP

SEQ ID NO: 43 - protein, 225 aa, Homo sapiens
MGLLGILCFLIFLGKTWGQEQTYVISAPKIFRVGASENIVIQVYGYTEAFDATISIKSYPDKKFSYSSGHVHLSSENKFQNSAILTIQPKQLPGGQNPVSYVYLEVVSKHFSKSKRMPITYDNGFLFIHTDKPVYTPDQSVKVRVYSLNDDLKPAKRETVLTFIDPEGSEVDMVEEIDHIGIISFPDFKIPSNPRYGMWTIKAKYKEDFSTTGTAYFEVKEYVLP

SEQ ID NO: 44 - protein, 1676 aa, Macaca fascicularis
MGLLGILCFLIFLGKTWGQEQTYVISAPKIFRVGASENIVIQVYGYTEAFDATISIKSYPDKKFSYSSGHVHLSSENKFQNSAVLTIQPKQLPGGQNQVSYVYLEVVSKHFSKSKKIPITYDNGFLFIHTDKPVYTPDQSVKVRVYSLNDDLKPAKRETVLTFIDPEGSEIDMVEEIDHIGIISFPDFKIPSNPRYGMWTIQAKYKEDFSTTGTAFFEVKEYVLPHFSVSVEPESNFIGYKNFKNFEITIKARYFYNKVVTEADVYITFGIREDLKDDQKEMMQTAMQNTMLINGIAEVTFDSETAVKELSYYSLEDLNNKYLYIAVTVIESTGGFSEEAEIPGIKYVLSPYKLNLVATPLFLKPGIPYSIKVQVKDALDQLVGGVPVTLNAQTIDVNQETSDLEPRKSVTRVDDGVASFVVNLPSGVTVLEFNVKTDAPDLPDENQAREGYRAIAYSSLSQSYLYIDWTDNHKALLVGEYLNIIVTPKSPYIDKITHYNYLILSKGKIIHFGTREKLSDASYQSINIPVTQNMVPSSRLLVYYIVTGEQTAELVSDSVWLNIEEKCGNQLQVHLSPDADTYSPGQTVSLNMVTGMDSWVALTAVDSAVYGVQRRAKKPLERVFQFLEKSDLGCGAGGGLNNANVFHLAGLTFLTNANADDSQENDEPCKEIIRPRRMLQEKIEEIAAKYKHLVVKKCCYDGVRINHDETCEQRAARISVGPRCVKAFTECCVVASQLRANNSHKDLQLGRLHMKTLLPVSKPEIRSYFPESWLWEVHLVPRRKQLQFALPDSVTTWEIQGVGISNSGICVADTIKAKVFKDVFLEMNIPYSVVRGEQVQLKGTVYNYRTSGMQFCVKMSAVEGICTSESPVIDHQGTKSSKCVRQKVEGSSNHLVTFTVLPLEIGLQNINFSLETSFGKEILVKSLRVVPEGVKRESYSGITLDPRGIYGTISRRKEFPYRIPLDLVPKTEIKRILSVKGLLVGEILSAVLSREGINILTHLPKGSAEAELMSVVPVFYVFHYLETGNHWNIFHSDPLIEKRNLEKKLKEGMVSIMSYRNADYSYSVWKGGSASTWLTAFALRVLGQVHKYVEQNQNSICNSLLWLVENYQLDNGSFKENSQYQPIKLQGTLPVEARENSLYLTAFTVIGIRKAFDICPLVKINTALIKADTFLLENTLPAQSTFTLAISAYALSLGDKTHPQFRSIVSALKREALVKGNPPIYRFWKDSLQHKDSSVPNTGTARMVETTAYALLTSLNLKDINYVNPIIKWLSEEQRYGGGFYSTQDTINAIEGLTEYSLLVKQLRLNMDIDVAYKHKGPLHNYKMTDKNFLGRPVEVLLNDDLVVSTGFGSGLATVHVTTVVHKTSTSEEVCSFYLKIDTQDIEASHYRGYGNSDYKRIVACASYKPSKEESSSGSSHAVMDISLPTGINANEEDLKALVEGVDQLFTDYQIKDGHVILQLNSIPSSDFLCVRFRIFELFEVGFLSPATFTVYEYHRPDKQCTMFYSTSNIKIQKVCEGATCKCIEADCGQMQKELDLTISAETRKQTACNPEIAYAYKVIITSITTENVFVKYKATLLDIYKTGEAVAEKDSEITFIKKVTCTNAELVKGRQYLIMGKEALQIKYNFTFRYIYPLDSLTWIEYWPRDTTCSSCQAFLANLDEFAEDIFLNGC

SEQ ID NO: 45 - protein, 6 aa, Artificial sequence
  An artificially synthesized sequence
SSYYMC

SEQ ID NO: 46 - protein, 6 aa, Artificial sequence
  An artificially synthesized sequence
NFYYIC

SEQ ID NO: 47 - protein, 6 aa, Artificial sequence
  An artificially synthesized sequence
SSYYMC

SEQ ID NO: 48 - protein, 6 aa, Artificial sequence
  An artificially synthesized sequence
SSYYMN

SEQ ID NO: 49 - protein, 6 aa, Artificial sequence
  An artificially synthesized sequence
SSYYMN

SEQ ID NO: 50 - protein, 5 aa, Artificial sequence
  An artificially synthesized sequence
DNTMT

SEQ ID NO: 51 - protein, 5 aa, Artificial sequence
  An artificially synthesized sequence
TYAMG

SEQ ID NO: 52 - protein, 5 aa, Artificial sequence
  An artificially synthesized sequence
GNAIN

SEQ ID NO: 53 - protein, 5 aa, Artificial sequence
  An artificially synthesized sequence
TYAMG

SEQ ID NO: 54 - protein, 6 aa, Artificial sequence
  An artificially synthesized sequence
SSYYVA

SEQ ID NO: 55 - protein, 17 aa, Artificial sequence
  An artificially synthesized sequence
CIYTGSGATYYASWAKG

SEQ ID NO: 56 - protein, 17 aa, Artificial sequence
  An artificially synthesized sequence
CIYTVSGYTYYASWAKG

SEQ ID NO: 57 - protein, 18 aa, Artificial sequence
  An artificially synthesized sequence
CIYAGSSGIIYYANWAKG

SEQ ID NO: 58 - protein, 16 aa, Artificial sequence
  An artificially synthesized sequence
MIYGSGATYYASWAKG

SEQ ID NO: 59 - protein, 16 aa, Artificial sequence
  An artificially synthesized sequence
MIYGSGATYYASWAKG

SEQ ID NO: 60 - protein, 16 aa, Artificial sequence
  An artificially synthesized sequence
IISFGGDAYYASWAKG

SEQ ID NO: 61 - protein, 16 aa, Artificial sequence
  An artificially synthesized sequence
TIDTGDNSFYANWAKG

SEQ ID NO: 62 - protein, 17 aa, Artificial sequence
  An artificially synthesized sequence
CIYTGSDTTYYATWAKG

SEQ ID NO: 63 - protein, 16 aa, Artificial sequence
  An artificially synthesized sequence
TIDTGDNSFYANWAKG

SEQ ID NO: 64 - protein, 17 aa, Artificial sequence
  An artificially synthesized sequence
AIYTGSGATYKASWAKG

SEQ ID NO: 65 - protein, 13 aa, Artificial sequence
  An artificially synthesized sequence
DGGYVTPTHAMYL

SEQ ID NO: 66 - protein, 9 aa, Artificial sequence
  An artificially synthesized sequence
DLHAGITNL

SEQ ID NO: 67 - protein, 13 aa, Artificial sequence
  An artificially synthesized sequence
YPTYGDGGHAFNL

SEQ ID NO: 68 - protein, 11 aa, Artificial sequence
  An artificially synthesized sequence
QIYSGDNNDNF

SEQ ID NO: 69 - protein, 11 aa, Artificial sequence
  An artificially synthesized sequence
QIYSGDNNDNF

SEQ ID NO: 70 - protein, 12 aa, Artificial sequence
  An artificially synthesized sequence
VGAGNIFWYFDL

SEQ ID NO: 71 - protein, 11 aa, Artificial sequence
  An artificially synthesized sequence
NDGSVYNLFNL

SEQ ID NO: 72 - protein, 4 aa, Artificial sequence
  An artificially synthesized sequence
GSGL

SEQ ID NO: 73 - protein, 11 aa, Artificial sequence
  An artificially synthesized sequence
NDGSVYNLFNL

SEQ ID NO: 74 - protein, 13 aa, Artificial sequence
  An artificially synthesized sequence
DGGYDYPTHAMHY

SEQ ID NO: 75 - protein, 11 aa, Artificial sequence
  An artificially synthesized sequence
QASQNIGSDLA

SEQ ID NO: 76 - protein, 11 aa, Artificial sequence
  An artificially synthesized sequence
QASQNIYSNLA

SEQ ID NO: 77 - protein, 13 aa, Artificial sequence
  An artificially synthesized sequence
QSSQSVYSSDYLS

SEQ ID NO: 78 - protein, 11 aa, Artificial sequence
  An artificially synthesized sequence
QASESISNWLA

SEQ ID NO: 79 - protein, 11 aa, Artificial sequence
  An artificially synthesized sequence
QASESISNWLA

SEQ ID NO: 80 - protein, 11 aa, Artificial sequence
  An artificially synthesized sequence
QASESIYSALA

SEQ ID NO: 81 - protein, 11 aa, Artificial sequence
  An artificially synthesized sequence
QASENIYSALS

SEQ ID NO: 82 - protein, 11 aa, Artificial sequence
  An artificially synthesized sequence
QASQNIYSLLA

SEQ ID NO: 83 - protein, 11 aa, Artificial sequence
  An artificially synthesized sequence
QASENIYSALS

SEQ ID NO: 84 - protein, 11 aa, Artificial sequence
  An artificially synthesized sequence
QASQNIGSSLA

SEQ ID NO: 85 - protein, 7 aa, Artificial sequence
  An artificially synthesized sequence
GASKLAS

SEQ ID NO: 86 - protein, 7 aa, Artificial sequence
  An artificially synthesized sequence
GASNLES

SEQ ID NO: 87 - protein, 7 aa, Artificial sequence
  An artificially synthesized sequence
EASKLAS

SEQ ID NO: 88 - protein, 7 aa, Artificial sequence
  An artificially synthesized sequence
RASTLAS

SEQ ID NO: 89 - protein, 7 aa, Artificial sequence
  An artificially synthesized sequence
RASTLAS

SEQ ID NO: 90 - protein, 7 aa, Artificial sequence
  An artificially synthesized sequence
SASTLAS

SEQ ID NO: 91 - protein, 7 aa, Artificial sequence
  An artificially synthesized sequence
YASTLAS

SEQ ID NO: 92 - protein, 7 aa, Artificial sequence
  An artificially synthesized sequence
HTSDLAS

SEQ ID NO: 93 - protein, 7 aa, Artificial sequence
  An artificially synthesized sequence
YASTLAS

SEQ ID NO: 94 - protein, 7 aa, Artificial sequence
  An artificially synthesized sequence
GASKTHS

SEQ ID NO: 95 - protein, 12 aa, Artificial sequence
  An artificially synthesized sequence
QCTFVGSSYGNA

SEQ ID NO: 96 - protein, 12 aa, Artificial sequence
  An artificially synthesized sequence
LQGYSYSNVDDA

SEQ ID NO: 97 - protein, 12 aa, Artificial sequence
  An artificially synthesized sequence
QGTYYSSGWYFA

SEQ ID NO: 98 - protein, 12 aa, Artificial sequence
  An artificially synthesized sequence
QQDYSSSNVDNT

SEQ ID NO: 99 - protein, 12 aa, Artificial sequence
  An artificially synthesized sequence
QQDYSSSNVDNT

SEQ ID NO: 100 - protein, 12 aa, Artificial sequence
  An artificially synthesized sequence
QQYYSSTNVHNS

SEQ ID NO: 101 - protein, 12 aa, Artificial sequence
  An artificially synthesized sequence
QQYYDINSVDNT

SEQ ID NO: 102 - protein, 13 aa, Artificial sequence
  An artificially synthesized sequence
QCTAYGSSDVGGT

SEQ ID NO: 103 - protein, 12 aa, Artificial sequence
  An artificially synthesized sequence
QQYYDINSVDNT

SEQ ID NO: 104 - protein, 12 aa, Artificial sequence
  An artificially synthesized sequence
QSTKVGSSYGNH

SEQ ID NO: 105 - protein, 1680 aa, Mus musculus
MGLWGILCLLIFLDKTWGQEQTYVISAPKILRVGSSENVVIQVHGYTEAFDATLSLKSYPDKKVTFSSGYVNLSPENKFQNAALLTLQPNQVPREESPVSHVYLEVVSKHFSKSKKIPITYNNGILFIHTDKPVYTPDQSVKIRVYSLGDDLKPAKRETVLTFIDPEGSEVDIVEENDYTGIISFPDFKIPSNPKYGVWTIKANYKKDFTTTGTAYFEIKEYVLPRFSVSIELERTFIGYKNFKNFEITVKARYFYNKVVPDAEVYAFFGLREDIKDEEKQMMHKATQAAKLVDGVAQISFDSETAVKELSYNSLEDLNNKYLYIAVTVTESSGGFSEEAEIPGVKYVLSPYTLNLVATPLFVKPGIPFSIKAQVKDSLEQAVGGVPVTLMAQTVDVNQETSDLETKRSITHDTDGVAVFVLNLPSNVTVLKFEIRTDDPELPEENQASKEYEAVAYSSLSQSYIYIAWTENYKPMLVGEYLNIMVTPKSPYIDKITHYNYLILSKGKIVQYGTREKLFSSTYQNINIPVTQNMVPSARLLVYYIVTGEQTAELVADAVWINIEEKCGNQLQVHLSPDEYVYSPGQTVSLDMVTEADSWVALSAVDRAVYKVQGNAKRAMQRVFQALDEKSDLGCGAGGGHDNADVFHLAGLTFLTNANADDSHYRDDSCKEILRSKRNLHLLRQKIEEQAAKYKHSVPKKCCYDGARVNFYETCEERVARVTIGPLCIRAFNECCTIANKIRKESPHKPVQLGRIHIKTLLPVMKADIRSYFPESWLWEIHRVPKRKQLQVTLPDSLTTWEIQGIGISDNGICVADTLKAKVFKEVFLEMNIPYSVVRGEQIQLKGTVYNYMTSGTKFCVKMSAVEGICTSGSSAASLHTSRPSRCVFQRIEGSSSHLVTFTLLPLEIGLHSINFSLETSFGKDILVKTLRVVPEGVKRESYAGVILDPKGIRGIVNRRKEFPYRIPLDLVPKTKVERILSVKGLLVGEFLSTVLSKEGINILTHLPKGSAEAELMSIAPVFYVFHYLEAGNHWNIFYPDTLSKRQSLEKKIKQGVVSVMSYRNADYSYSMWKGASASTWLTAFALRVLGQVAKYVKQDENSICNSLLWLVEKCQLENGSFKENSQYLPIKLQGTLPAEAQEKTLYLTAFSVIGIRKAVDICPTMKIHTALDKADSFLLENTLPSKSTFTLAIVAYALSLGDRTHPRFRLIVSALRKEAFVKGDPPIYRYWRDTLKRPDSSVPSSGTAGMVETTAYALLASLKLKDMNYANPIIKWLSEEQRYGGGFYSTQDTINAIEGLTEYSLLLKQIHLDMDINVAYKHEGDFHKYKVTEKHFLGRPVEVSLNDDLVVSTGYSSGLATVYVKTVVHKISVSEEFCSFYLKIDTQDIEASSHFRLSDSGFKRIIACASYKPSKEESTSGSSHAVMDISLPTGIGANEEDLRALVEGVDQLLTDYQIKDGHVILQLNSIPSRDFLCVRFRIFELFQVGFLNPATFTVYEYHRPDKQCTMIYSISDTRLQKVCEGAACTCVEADCAQLQAEVDLAISADSRKEKACKPETAYAYKVRITSATEENVFVKYTATLLVTYKTGEAADENSEVTFIKKMSCTNANLVKGKQYLIMGKEVLQIKHNFSFKYIYPLDSSTWIEYWPTDTTCPSCQAFVENLNNFAEDLFLNSCE

SEQ ID NO: 106 - protein, 123 aa, Artificial sequence [sequence omitted]

SEQ ID NO: 107 - protein, 123 aa, Artificial sequence
  An artificially synthesized sequence
QVQLVESGGGLVQPGRSLRLSCAASGFTVHSSYYMAWVRQAPGKGLEWVGAIFTGSGAEYKAEWVKGRFTISRDNSKNTLYLQMNSLRAEDTAVYYCASDAGYDYPTHAMHYWGRGTLVTVSS

SEQ ID NO: 108 - protein, 123 aa, Artificial sequence
  An artificially synthesized sequence
QVQLVESGGGLVQPGRSLRLSCAASGFTVHSSYYMAWVRQAPGKGLEWVGAIFTGSGAEYKAEWAKGRVTISKDTSKNQVVLTMTNMDPVDTATYYCASDAGYDYPTHAMHYWGRGTLVTVSS

SEQ ID NO: 109 - protein, 123 aa, Artificial sequence
  An artificially synthesized sequence
QVQLVESGGGLVQPGGSLRLSCAASGFTVHSSYYMAWVRQAPGKGLEWVGAIFTGSGAEYKAEWAKGRVTISKDTSKNQVVLTMTNMDPVDTATYYCASDAGYDYPTHAMHYWGQGTLVTVSS

SEQ ID NO: 110 - protein, 123 aa, Artificial sequence
  An artificially synthesized sequence
QVQLVESGGGLVQPGGSLRLSCAASGFTVHSSYYMAWVRQAPGKGLEWVSGIFTGSGATYKAEWAKGRVTISKDTSKNQVVLTMTNMDPVDTATYYCASDAGYDYPTHAMHYWGQGTLVTVSS

SEQ ID NO: 111 - protein, 110 aa, Artificial sequence [sequence omitted]

SEQ ID NO: 112 - protein, 110 aa, Artificial sequence
  An artificially synthesized sequence
DIQMTQSPSSLSASVGDRVTITCRASQGISSSLAWYQQKPGQAPRLLIYGASETESGVPSRFSGSGSGTDFTLTISSLQPEDFATYYCQNTKVGSSYGNTFGGGTKVEIK

SEQ ID NO: 113 - protein, 110 aa, Artificial sequence
  An artificially synthesized sequence
DIQMTQSPSSLSASVGDRVTITCRASQGISSSLAWYQQKPGQAPRLLIYGASTTQSGVPSRFSGSGSGTDFTLTISSLQPEDFATYYCQNTKVGSSYGNTFGGGTKVEIK

SEQ ID NO: 114 - protein, 328 aa, Artificial sequence
  An artificially synthesized sequence
ASTKGPSVFPLAPSSKSTSGGTAALGCLVKDYFPEPVTVSWNSGALTSGVHTFPAVLQSSGLYSLSSVVTVPSSSLGTQTYICNVNHKPSNTKVDKKVEPKSCDKTHTCPPCPAPELRRGPKVFLFPPKPKDTLMISRTPEVTCVVVDVSHEDPEVKFNWYVDGVEVHNAKTKPREEQYNSTYRVVSVLTVLHQDWLNGKEYKCKVSNKGLPSSIEKTISKAKGQPREPQVYTLPPSREEMTKNQVSLTCLVKGFYPSDIAVEWESNGQPENNYKTTPPVLDSDGSFFLYSKLTVDKSRWQQGNVFSCSVLHEALHAHYTRKELSLSP

SEQ ID NO: 115 - protein, 325 aa, Artificial sequence
  An artificially synthesized sequence
ASTKGPSVFPLAPCSRSTSGGTAALGCLVKDYFPEPVTVSWNSGALTSGVHTFPAVLQSSGLYSLSSVVTVPSSSLGTKTYTCNVDHKPSNTKVDKRVESKYGPPCPPCPAPEFRRGPKVFLFPPKPKDTLMISRTPEVTCVVVDVSHEDPEVKFNWYVDGVEVHNAKTKPREEQYNSTYRVVSVLTVLHQDWLNGKEYKCKVSNKGLPSSIEKTISKAKGQPREPQVYTLPPSREEMTKNQVSLTCLVKGFYPSDIAVEWESNGQPENNYKTTPPVLDSDGSFFLYSKLTVDKSRWQQGNVFSCSVLHEALHAHYTRKELSLSP

SEQ ID NO: 116 - protein, 325 aa, Artificial sequence
  An artificially synthesized sequence
ASTKGPSVFPLAPCSRSTSGGTAALGCLVKDYFPEPVTVSWNSGALTSGVHTFPAVLQSSGLYSLSSVVTVPSSSLGTKTYTCNVDHKPSNTKVDKRVESKYGPPCPPCPAPEFRRGPKVFLFPPKPKDTLMISRTPEVTCVVVDVSHEDPEVKFNWYVDGVEVHNAKTKPREEQYNSTYRVVSVLTVLHQDWLNGKEYKCKVSNKGLPSSIEKTISKAKGQPREPQVYTLPPSREEMTKNQVSLTCLVKGFYPSDIAVEWESNGQPENNYKTTPPVLDSDGSFFLYSRLTVDKSRWQQGNVFSCSVLHEALHAHYTRKELSLSP

SEQ ID NO: 117 - protein, 6 aa, Artificial sequence
  An artificially synthesized sequence
SSYYMA

SEQ ID NO: 118 - protein, 17 aa, Artificial sequence
  An artificially synthesized sequence
AIFTGSGAEYKAEWAKG

SEQ ID NO: 119 - protein, 17 aa, Artificial sequence
  An artificially synthesized sequence
AIFTGSGAEYKAEWVKG

SEQ ID NO: 120 - protein, 17 aa, Artificial sequence
  An artificially synthesized sequence
GIFTGSGATYKAEWAKG

SEQ ID NO: 121 - protein, 13 aa, Artificial sequence
  An artificially synthesized sequence
DAGYDYPTHAMHY

SEQ ID NO: 122 - protein, 11 aa, Artificial sequence
  An artificially synthesized sequence
RASQGISSSLA

SEQ ID NO: 123 - protein, 7 aa, Artificial sequence
  An artificially synthesized sequence
GASETES

SEQ ID NO: 124 - protein, 7 aa, Artificial sequence
  An artificially synthesized sequence
GASTTQS

SEQ ID NO: 125 - protein, 12 aa, Artificial sequence
  An artificially synthesized sequence
QNTKVGSSYGNT

SEQ ID NO: 126 - protein, 6 aa, Artificial sequence
  An artificially synthesized sequence
  misc_feature (5)..(5): Xaa is Met or Val
  misc_feature (6)..(6): Xaa is Cys or Ala
SSYYXX

SEQ ID NO: 127 - protein, 17 aa, Artificial sequence
  An artificially synthesized sequence
  misc_feature (1)..(1): Xaa is Cys, Ala or Gly
  misc_feature (3)..(3): Xaa is Tyr or Phe
  misc_feature (9)..(9): Xaa is Thr, Asp or Glu
  misc_feature (11)..(11): Xaa is Tyr, Lys or Gln
  misc_feature (13)..(13): Xaa is Ser, Asp or Glu
  misc_feature (15)..(15): Xaa is Ala or Val
XIXTGSGAXYXAXWXKG

SEQ ID NO: 128 - protein, 13 aa, Artificial sequence
  An artificially synthesized sequence
  misc_feature (2)..(2): Xaa is Gly or Ala
  misc_feature (5)..(5): Xaa is Val, Gln or Asp
  misc_feature (6)..(6): Xaa is Thr or Tyr
  misc_feature (12)..(12): Xaa is Tyr or His
  misc_feature (13)..(13): Xaa is Leu or Tyr
DXGYXXPTHAMXX

SEQ ID NO: 129 - protein, 11 aa, Artificial sequence
  An artificially synthesized sequence
  misc_feature (1)..(1): Xaa is Gln or Arg
  misc_feature (5)..(5): Xaa is Asn, Gln or Gly
  misc_feature (7)..(7): Xaa is Gly or Ser
  misc_feature (9)..(9): Xaa is Asp, Lys or Ser
XASQXIXSXLA

SEQ ID NO: 130 - protein, 7 aa, Artificial sequence
  An artificially synthesized sequence
  misc_feature (4)..(4): Xaa is Lys, Glu or Thr
  misc_feature (5)..(5): Xaa is Leu or Thr
  misc_feature (6)..(6): Xaa is Ala, His, Glu or Gln
GASXXXS

SEQ ID NO: 131 - protein, 12 aa, Artificial sequence
  An artificially synthesized sequence
  misc_feature (2)..(2): Xaa is Ser, Cys, Asn or Thr
  misc_feature (4)..(4): Xaa is Phe or Lys
  misc_feature (12)..(12): Xaa is Ala, Thr or His
QXTXVGSSYGNX

SEQ ID NO: 132 - protein, 30 aa, Artificial sequence
  An artificially synthesized sequence
QVQLVESGGGLVQPGGSLRLSCAASGFTSH

SEQ ID NO: 133 - protein, 30 aa, Artificial sequence
  An artificially synthesized sequence
QVQLVESGGGLVQPGRSLRLSCAASGFTVH

SEQ ID NO: 134 - protein, 30 aa, Artificial sequence
  An artificially synthesized sequence
QVQLVESGGGLVQPGGSLRLSCAASGFTVH

SEQ ID NO: 135 - protein, 14 aa, Artificial sequence
  An artificially synthesized sequence
WVRQAPGKGLEWVG

SEQ ID NO: 136 - protein, 14 aa, Artificial sequence
  An artificially synthesized sequence
WVRQAPGKGLEWVS

SEQ ID NO: 137 - protein, 32 aa, Artificial sequence
  An artificially synthesized sequence
RFTISKDTSKNQVVLTMTNMDPVDTATYYCAS

SEQ ID NO: 138 - protein, 32 aa, Artificial sequence
  An artificially synthesized sequence
RVTISKDTSKNQVVLTMTNMDPVDTATYYCAS

SEQ ID NO: 139 - protein, 32 aa, Artificial sequence
  An artificially synthesized sequence
RFTISRDNSKNTLYLQMNSLRAEDTAVYYCAS

SEQ ID NO: 140 - protein, 11 aa, Artificial sequence
  An artificially synthesized sequence
WGQGTLVTVSS

SEQ ID NO: 141 - protein, 11 aa, Artificial sequence
  An artificially synthesized sequence
WGRGTLVTVSS

SEQ ID NO: 142 - protein, 23 aa, Artificial sequence
  An artificially synthesized sequence
DVVMTQSPSSLSASVGDRVTITC

SEQ ID NO: 143 - protein, 23 aa, Artificial sequence
  An artificially synthesized sequence
DIQMTQSPSSLSASVGDRVTITC

SEQ ID NO: 144 - protein, 15 aa, Artificial sequence
  An artificially synthesized sequence
WYQQKPGQAPRLLIY

SEQ ID NO: 145 - protein, 15 aa, Artificial sequence
  An artificially synthesized sequence
WYQQKPGKAPKLLIY

SEQ ID NO: 146 - protein, 32 aa, Artificial sequence
  An artificially synthesized sequence
GVPSRFSGSGSGTDFTLTISSLQPEDVATYYC

SEQ ID NO: 147 - protein, 32 aa, Artificial sequence
  An artificially synthesized sequence
GVPSRFSGSGSGTDFTLTISSLQPEDFATYYC

SEQ ID NO: 148 - protein, 10 aa, Artificial sequence
  An artificially synthesized sequence
FGGGTKVEIK

SEQ ID NO: 149 - protein, 448 aa, Artificial sequence
  An artificially synthesized sequence
QVQLVQSGAEVKKPGASVKVSCKASGHIFSNYWIQWVRQAPGQGLEWMGEILPGSGHTEYTENFKDRVTMTRDTSTSTVYMELSSLRSEDTAVYYCARYFFGSSPNWYFDVWGQGTLVTVSSASTKGPSVFPLAPCSRSTSESTAALGCLVKDYFPEPVTVSWNSGALTSGVHTFPAVLQSSGLYSLSSVVTVPSSNFGTQTYTCNVDHKPSNTKVDKTVERKCCVECPPCPAPPVAGPSVFLFPPKPKDTLMISRTPEVTCVVVDVSQEDPEVQFNWYVDGVEVHNAKTKPREEQFNSTYRVVSVLTVLHQDWLNGKEYKCKVSNKGLPSSIEKTISKAKGQPREPQVYTLPPSQEEMTKNQVSLTCLVKGFYPSDIAVEWESNGQPENNYKTTPPVLDSDGSFFLYSRLTVDKSRWQEGNVFSCSVLHEALHSHYTQKSLSLSLGK

SEQ ID NO: 150 - protein, 214 aa, Artificial sequence [sequence omitted]